European Patent Application EP 4 647 443 A1, published November 12, 2025. Title: Therapeutic variable domain of heavy chain (VHH) antibody fusions co-neutralizing alpha- and gamma-hemolysins from Staphylococcus aureus. Applicant: Max-Planck-Gesellschaft zur Foerderung der Wissenschaften e.V. The sequence listing filed with the application follows.

SEQUENCE LISTING (197 sequences)

SEQ ID NO: 1 - protein, 280 aa, synthetic construct
  source 1..280: note = Hlg-A (UniProt P0A074 (30-309))
ENKIEDIGQGAEIIKRTQDITSKRLAITQNIQFDFVKDKKYNKDALVVKMQGFISSRTTYSDLKKYPYIKRMIWPFQYNISLKTKDSNVDLINYLPKNKIDSADVSQKLGYNIGGNFQSAPSIGGSGSFNYSKTISYNQKNYVTEVESQNSKGVKWGVKANSFVTPNGQVSAYDQYLFAQDPTGPAARDYFVPDNQLPPLIQSGFNPSFITTLSHERGKGDKSEFEITYGRNMDATYAYVTRHRLAVDRKHDAFKNRNVTVKYEVNWKTHEVKIKSITPK

SEQ ID NO: 2 - protein, 299 aa, synthetic construct
  source 1..299: note = Hlg-B (UniProt P0A077 (36-325))
EGKITPVSVKKVDDKVTLYKTTATADSDKFKISQILTFNFIKDKSYDKDTLVLKATGNINSGFVKPNPNDYDFSKLYWGAKYNVSISSQSNDSVNVVDYAPKNQNEEFQVQNTLGYTFGGDISISNGLSGGLNGNTAFSETINYKQESYRTTLSRNTNYKNVGWGVEAHKIMNNGWGPYGRDSFHPTYGNELFLAGRQSSAYAGQNFIAQHQMPLLSRSNFNPEFLSVLSHRQDGAKKSKITVTYQREMDLYQIRWNGFYWAGANYKNFKTRTFKSTYEIDWENHKVKLLDTKETENNK

SEQ ID NO: 3 - protein, 286 aa, synthetic construct
  source 1..286: note = Hlg-C (UniProt Q07227 (30-315))
ANDTEDIGKGSDIEIIKRTEDKTSNKWGVTQNIQFDFVKDKKYNKDALILKMQGFISSRTTYYNYKKTNHVKAMRWPFQYNIGLKTNDKYVSLINYLPKNKIESTNVSQTLGYNIGGNFQSAPSLGGNGSFNYSKSISYTQQNYVSEVEQQNSKSVLWGVKANSFATESGQKSAFDSDLFVGYKPHSKDPRDYFVPDSELPPLVQSGFNPSFIATVSHEKGSSDTSEFEITYGRNMDVTHAIKRSTHYGNSYLDGHRVHNAFVNRNYTVKYEVNWKTHEIKVKGQN

SEQ ID NO: 4 - protein, 293 aa, synthetic construct
  source 1..293: note = Hla (UniProt P09616 (27-319))
ADSDINIKTGTTDIGSNTTVKTGDLVTYDKENGMHKKVFYSFIDDKNHNKKLLVIRTKGTIAGQYRVYSEEGANKSGLAWPSAFKVQLQLPDNEVAQISDYYPRNSIDTKEYMSTLTYGFNGNVTGDDTGKIGGLIGANVSIGHTLKYVQPDFKTILESPTDKKVGWKVIFNNMVNQNWGPYDRDSWNPVYGNQLFMKTRNGSMKAADNFLDPNKASSLLSSGFSPDFATVITMDRKASKQQTNIDVIYERVRDDYQLHWTSTNWKGTNTKDKWTDRSSERYKIDWEKEEMTN

SEQ ID NO: 5 - protein, 126 aa, synthetic construct
  source 1..126: note = Bm29C02
QVQLVESGGGLVQPGGSLRLSCTASGFTLDDWAIGWFRQAPGKEREGVSCTSSRERSSYYRDSVKGRFTISRDSTSNTVYLQMNELTLEDTAVYYCAADPQPYPCSLGQLGRYTTWGQGTQVTVSS

SEQ ID NO: 6 - protein, 12 aa, synthetic construct
  source 1..12: note = CDR1
GFTLDDWAIGWF

SEQ ID NO: 7 - protein, 15 aa, synthetic construct
  source 1..15: note = CDR2
GVSCTSSRERSSYYR

SEQ ID NO: 8 - protein, 20 aa, synthetic construct
  source 1..20: note = CDR3
AADPQPYPCSLGQLGRYTTW

SEQ ID NO: 9 - protein, 126 aa, synthetic construct
  source 1..126: note = Bm29H04
QVQLVESGGGLVQPGGSLRLSCTASGVSLDDFAIGWFRQAPGKEREGVSCSSSRDRSEYYRDSVKGRFTISRDSQKNTVDLQMNSLTIEDTAVYYCAADPQPYPCSVGSLDRYNSWGQGTLVTVSS

SEQ ID NO: 10 - protein, 12 aa, synthetic construct
  source 1..12: note = CDR1
GVSLDDFAIGWF

SEQ ID NO: 11 - protein, 15 aa, synthetic construct
  source 1..15: note = CDR2
GVSCSSSRDRSEYYR

SEQ ID NO: 12 - protein, 20 aa, synthetic construct
  source 1..20: note = CDR3
AADPQPYPCSVGSLDRYNSW

SEQ ID NO: 13 - protein, 126 aa, synthetic construct
  source 1..126: note = Bm29E06
QVQLVESGGGLVQPGGSLRLSCTASGVSLYDFAVGWFRQAPGKEREGVSCSSSRDRSEYYRDSVKGRFDIVRDNLKNIIYLQMDNLTIEDTAVYFCAADSQPYPCSLGSLERYDSWGQGTQVTVSS

SEQ ID NO: 14 - protein, 12 aa, synthetic construct
  source 1..12: note = CDR1
GVSLYDFAVGWF

SEQ ID NO: 15 - protein, 15 aa, synthetic construct
  source 1..15: note = CDR2
GVSCSSSRDRSEYYR

SEQ ID NO: 16 - protein, 20 aa, synthetic construct
  source 1..20: note = CDR3
AADSQPYPCSLGSLERYDSW

SEQ ID NO: 17 - protein, 126 aa, synthetic construct
  source 1..126: note = Bm29F05
QVQLVESGGGLVQPGGSLRLSCTASGVSLYDFAVGWWRQAPGKEREGVSCTSSRDRSEYYRDSVKGRFTIVRDNLKNTIYLQMDSLTIEDTAVYFCAADSQPYPCSLGSLERYDSWGQGIQVTVSS

SEQ ID NO: 18 - protein, 12 aa, synthetic construct
  source 1..12: note = CDR1
GVSLYDFAVGWW

SEQ ID NO: 19 - protein, 15 aa, synthetic construct
  source 1..15: note = CDR2
GVSCTSSRDRSEYYR

SEQ ID NO: 20 - protein, 20 aa, synthetic construct
  source 1..20: note = CDR3
AADSQPYPCSLGSLERYDSW

SEQ ID NO: 21 - protein, 122 aa, synthetic construct
  source 1..122: note = Bm29B04
QVQLVESGGGLVQAGGSLRLSCAASGFTFDDYVIGWFRQAPGKEREAVACISNGDGVANVPNSMKGRFTISSDSAKNTVHLRADSLKADDTGVYYCAAVKERLCVHEGMEYWGKGTQVTVSS

SEQ ID NO: 22 - protein, 12 aa, synthetic construct
  source 1..12: note = CDR1
GFTFDDYVIGWF

SEQ ID NO: 23 - protein, 15 aa, synthetic construct
  source 1..15: note = CDR2
AVACISNGDGVANVP

SEQ ID NO: 24 - protein, 16 aa, synthetic construct
  source 1..16: note = CDR3
AAVKERLCVHEGMEYW

SEQ ID NO: 25 - protein, 122 aa, synthetic construct
  source 1..122: note = Bm29B05
QVQLVESGGGLVQAGGSLRLSCAASGFTFDDYVIGWFRQAPGKEREAVACISNGDGVTNYPNSMRGRFTISSDSAKNTVYLQTDSLKPDDTGVYYCATAKERLCVQGGMEYWGKGTLVTVSS

SEQ ID NO: 26 - protein, 12 aa, synthetic construct
  source 1..12: note = CDR1
GFTFDDYVIGWF

SEQ ID NO: 27 - protein, 15 aa, synthetic construct
  source 1..15: note = CDR2
AVACISNGDGVTNYP

SEQ ID NO: 28 - protein, 16 aa, synthetic construct
  source 1..16: note = CDR3
ATAKERLCVQGGMEYW

SEQ ID NO: 29 - protein, 123 aa, synthetic construct
  source 1..123: note = Bm29D07
QVQLVESGGGLVQPGGSLRLSCTASSIIVSYYAIGWFRQAPGKGREGVSRITVPAGNLYYADSVKGRFSITRDDVKNTVYLQMNSFQVEDTATYYCAVSYGDSWVDPSYVDHWGQGIQVTVSS

SEQ ID NO: 30 - protein, 12 aa, synthetic construct
  source 1..12: note = CDR1
SIIVSYYAIGWF

SEQ ID NO: 31 - protein, 15 aa, synthetic construct
  source 1..15: note = CDR2
GVSRITVPAGNLYYA

SEQ ID NO: 32 - protein, 17 aa, synthetic construct
  source 1..17: note = CDR3
AVSYGDSWVDPSYVDHW

SEQ ID NO: 33 - protein, 121 aa, synthetic construct
  source 1..121: note = Bm31D04
QVQLVESGGGLVQPGGSLRLSCAASGIIFDFYDMGWYRQAPGKQRELVAGISISGSTTYADSVKGRFTISRDNAKNTIYLQMNSLKPEDTAVYYCNAHHVDSDYLRGYDYFGQGTQVTVSS

SEQ ID NO: 34 - protein, 12 aa, synthetic construct
  source 1..12: note = CDR1
GIIFDFYDMGWY

SEQ ID NO: 35 - protein, 14 aa, synthetic construct
  source 1..14: note = CDR2
LVAGISISGSTTYA

SEQ ID NO: 36 - protein, 16 aa, synthetic construct
  source 1..16: note = CDR3
NAHHVDSDYLRGYDYF

SEQ ID NO: 37 - protein, 121 aa, synthetic construct
  source 1..121: note = Bm31G03
QVQLVESGGGLVQAGGSLRLSCAASGIIFSFYDMGWYRQAPGKQREVVATISISGRTTYADSVKGRFTISRDDAKNTVYLQMNSLKPEDTAVYICNAQHVDSDYLAGYDYFGQGTQVTVSS

SEQ ID NO: 38 - protein, 12 aa, synthetic construct
  source 1..12: note = CDR1
GIIFSFYDMGWY

SEQ ID NO: 39 - protein, 14 aa, synthetic construct
  source 1..14: note = CDR2
VVATISISGRTTYA

SEQ ID NO: 40 - protein, 16 aa, synthetic construct
  source 1..16: note = CDR3
NAQHVDSDYLAGYDYF

SEQ ID NO: 41 - protein, 121 aa, synthetic construct
  source 1..121: note = Bm31G04
QVQLVESGGGLVQPGGSLRLSCAASGITFTFYDMGWYRQAPGKQRELVATISISSSTTYADSVKGRFTISRDNAKNTVYLQMNSLKPEDTAVYYCNAQHVDSDYLAGYDYFGQGTQVTVSS

SEQ ID NO: 42 - protein, 12 aa, synthetic construct
  source 1..12: note = CDR1
GITFTFYDMGWY

SEQ ID NO: 43 - protein, 14 aa, synthetic construct
  source 1..14: note = CDR2
LVATISISSSTTYA

SEQ ID NO: 44 - protein, 16 aa, synthetic construct
  source 1..16: note = CDR3
NAQHVDSDYLAGYDYF

SEQ ID NO: 45 - protein, 126 aa, synthetic construct
  source 1..126: note = Bm31F09
QVQLVESGGALVQPGGSLRLSCAASGFTFDDYVMSWVRQAPGTGLEWVSSIHTASSDTYYADSVKDRFTISTDNAKNTLYLQMNSLKPEDTAVYYCAADKAPLTIATMTRDEYDYWGQGTQVTVSS

SEQ ID NO: 46 - protein, 12 aa, synthetic construct
  source 1..12: note = CDR1
GFTFDDYVMSWV

SEQ ID NO: 47 - protein, 15 aa, synthetic construct
  source 1..15: note = CDR2
WVSSIHTASSDTYYA

SEQ ID NO: 48 - protein, 20 aa, synthetic construct
  source 1..20: note = CDR3
AADKAPLTIATMTRDEYDYW

SEQ ID NO: 49 - protein, 126 aa, synthetic construct
  source 1..126: note = Bm31G12
QVQLVESGGGLVQPGGSLRLSCAAAGFTVDDYVMSWVRQVPGKGREWVSSIHSYSSDTYYADSVKGRFTISTDNAKNTLYLQMNSLKPEDTAVYYCAADKDPLTIATMTRYEYDYWGQGTQVTVSS

SEQ ID NO: 50 - protein, 12 aa, synthetic construct
  source 1..12: note = CDR1
GFTVDDYVMSWV

SEQ ID NO: 51 - protein, 15 aa, synthetic construct
  source 1..15: note = CDR2
WVSSIHSYSSDTYYA

SEQ ID NO: 52 - protein, 20 aa, synthetic construct
  source 1..20: note = CDR3
AADKDPLTIATMTRYEYDYW

SEQ ID NO: 53 - protein, 128 aa, synthetic construct
  source 1..128: note = Bm31A09
QVQLVQSGGGLVQAGGSLRLSCAASGSTGSIYVMGWFRQAPGKQRELVASITRGEGSANYADSVKGRFTISRDNAKNTLYLQMNSLKPEDTAVYYCHADTGLGDYSDYAPHGYKYDYWGQGTQVTVSS

SEQ ID NO: 54 - protein, 12 aa, synthetic construct
  source 1..12: note = CDR1
GSTGSIYVMGWF

SEQ ID NO: 55 - protein, 15 aa, synthetic construct
  source 1..15: note = CDR2
LVASITRGEGSANYA

SEQ ID NO: 56 - protein, 22 aa, synthetic construct
  source 1..22: note = CDR3
HADTGLGDYSDYAPHGYKYDYW

SEQ ID NO: 57 - protein, 128 aa, synthetic construct
  source 1..128: note = Bm31D02
QVQLVESGGGLVQAGGSLRLSCAASGSTGSIYVMGWFRQAPGKQRELVASITRGEGSANYADSVKGRFTISRDNAKNTLYLQMNSLKPEDTAVYYCHADTGLGDYSDYAPHGYKYDYWGQGTQVTVSS

SEQ ID NO: 58 - protein, 12 aa, synthetic construct
  source 1..12: note = CDR1
GSTGSIYVMGWF

SEQ ID NO: 59 - protein, 15 aa, synthetic construct
  source 1..15: note = CDR2
LVASITRGEGSANYA

SEQ ID NO: 60 - protein, 22 aa, synthetic construct
  source 1..22: note = CDR3
HADTGLGDYSDYAPHGYKYDYW

SEQ ID NO: 61 - protein, 123 aa, synthetic construct
  source 1..123: note = Bm31A04
QVQLVQSGGGLVQPGGSLRLSCAASESISNIYVMGWFRQAPGKQRELVAAITSSNNTNYADSVKGRFTISRDNAKNTVYLQMNSLKPEDTAVYYCNADWGLGGYSDYGEYDYWGQGTQVTVSS

SEQ ID NO: 62 - protein, 12 aa, synthetic construct
  source 1..12: note = CDR1
ESISNIYVMGWF

SEQ ID NO: 63 - protein, 14 aa, synthetic construct
  source 1..14: note = CDR2
LVAAITSSNNTNYA

SEQ ID NO: 64 - protein, 18 aa, synthetic construct
  source 1..18: note = CDR3
NADWGLGGYSDYGEYDYW

SEQ ID NO: 65 - protein, 124 aa, synthetic construct
  source 1..124: note = Bm31A08
QVQLVESGGGLAQPGGSLTLSCAASGVVWSKYVMSWVRQVPEKGFEWVSGIKSDGSDTYYADSVKGRFTVSGDLAKKTVYLQLNSLKPEDTALYYCVLEYGTSWPPRVEEYDYWGQGTQVTVSS

SEQ ID NO: 66 - protein, 12 aa, synthetic construct
  source 1..12: note = CDR1
GVVWSKYVMSWV

SEQ ID NO: 67 - protein, 15 aa, synthetic construct
  source 1..15: note = CDR2
WVSGIKSDGSDTYYA

SEQ ID NO: 68 - protein, 18 aa, synthetic construct
  source 1..18: note = CDR3
VLEYGTSWPPRVEEYDYW

SEQ ID NO: 69 - protein, 121 aa, synthetic construct
  source 1..121: note = Bm31B04
QVQLVESGGGLVQPGGSLRLSCAASGSSFSIYGMSWYRQAPGNQRELVALINVGDWTTYADSVKGRFTISRDSAKNTVYLQMNSLKPEDTAVYYCKADLSVSGSSFIRTYWGQGTQVTVSS

SEQ ID NO: 70 - protein, 12 aa, synthetic construct
  source 1..12: note = CDR1
GSSFSIYGMSWY

SEQ ID NO: 71 - protein, 14 aa, synthetic construct
  source 1..14: note = CDR2
LVALINVGDWTTYA

SEQ ID NO: 72 - protein, 16 aa, synthetic construct
  source 1..16: note = CDR3
KADLSVSGSSFIRTYW

SEQ ID NO: 73 - protein, 126 aa, synthetic construct
  source 1..126: note = Bm32A03
QVQLVESGGALVQTGGSLRLSCVTSGSISSIYAMPWFRQAPGKEREFVAAISWHTNLAYYADSVKGRFTISKDNAKNTVYLQMDSLKPEDTATYYCNVPSKEEYDRTSYYPTGGSWGQGTQVTVSS

SEQ ID NO: 74 - protein, 12 aa, synthetic construct
  source 1..12: note = CDR1
GSISSIYAMPWF

SEQ ID NO: 75 - protein, 15 aa, synthetic construct
  source 1..15: note = CDR2
FVAAISWHTNLAYYA

SEQ ID NO: 76 - protein, 20 aa, synthetic construct
  source 1..20: note = CDR3
NVPSKEEYDRTSYYPTGGSW

SEQ ID NO: 77 - protein, 126 aa, synthetic construct
  source 1..126: note = Bm32B07
QVQLVESGGGLVQTGGSLRLSCATSGRISSIYAMPWFRQAPGKEREFVAAISWHTDLAYYADSVKGRFTISKDNAKNTVYLQMNSLKPEDTAVYYCNIPSKEEYDRNYYYPTGGSWGQGTQVTVSS

SEQ ID NO: 78 - protein, 12 aa, synthetic construct
  source 1..12: note = CDR1
GRISSIYAMPWF

SEQ ID NO: 79 - protein, 15 aa, synthetic construct
  source 1..15: note = CDR2
FVAAISWHTDLAYYA

SEQ ID NO: 80 - protein, 20 aa, synthetic construct
  source 1..20: note = CDR3
NIPSKEEYDRNYYYPTGGSW

SEQ ID NO: 81 - protein, 126 aa, synthetic construct
  source 1..126: note = Bm32D01
QVQLVESGGGLVQTGGSLRLSCATSGRISSIYAMPWFRQAPGKEREFVAAISWHTDLTYYADSVKDRFTISKDNAKATVYLQMNNLQPEDTAVYYCNVPSKEQYDRTSYYPTGGSWGQGTQVTVSS

SEQ ID NO: 82 - protein, 12 aa, synthetic construct
  source 1..12: note = CDR1
GRISSIYAMPWF

SEQ ID NO: 83 - protein, 15 aa, synthetic construct
  source 1..15: note = CDR2
FVAAISWHTDLTYYA

SEQ ID NO: 84 - protein, 20 aa, synthetic construct
  source 1..20: note = CDR3
NVPSKEQYDRTSYYPTGGSW

SEQ ID NO: 85 - protein, 125 aa, synthetic construct
  source 1..125: note = Bm32A08
QVQLVESGGGLVQAGGSLRVSCAASGDWFIINSMAWFRQAPGKQREQVATISHGGIPRYADSVKGRFTISRDNSKGAVYLQMNNLKSDDTAMYVCAAGGLDYGFPDPTPEEFDYWGRGTQVTVSS

SEQ ID NO: 86 - protein, 12 aa, synthetic construct
  source 1..12: note = CDR1
GDWFIINSMAWF

SEQ ID NO: 87 - protein, 14 aa, synthetic construct
  source 1..14: note = CDR2
QVATISHGGIPRYA

SEQ ID NO: 88 - protein, 20 aa, synthetic construct
  source 1..20: note = CDR3
AAGGLDYGFPDPTPEEFDYW

SEQ ID NO: 89 - protein, 125 aa, synthetic construct
  source 1..125: note = Bm32F03
QVQLVESGGGLVQAGGSLRVSCAASGDWFIINSMAWFRQAPGKQREQVATISHGGIPRYADSVKGRFTISRDDSKDAVYLQMNNLKSDDTAMYVCAAGGLDYGFPDPTPEEFDYWGRGTQVTVSS

SEQ ID NO: 90 - protein, 12 aa, synthetic construct
  source 1..12: note = CDR1
GDWFIINSMAWF

SEQ ID NO: 91 - protein, 14 aa, synthetic construct
  source 1..14: note = CDR2
QVATISHGGIPRYA

SEQ ID NO: 92 - protein, 20 aa, synthetic construct
  source 1..20: note = CDR3
AAGGLDYGFPDPTPEEFDYW

SEQ ID NO: 93 - protein, 123 aa, synthetic construct
  source 1..123: note = VHH_Ma7A07
QVQLVESGGGLVQPGGSLRLSCAASGFTLGDYTLGWFRQAPGKQREGVSSIASSALSIYIADSVKGRFTISRDDAKNTIYLHMNNLKPEDTGVYYCARGVDSWRWVPSAMDLWGKGTLVTVSS

SEQ ID NO: 94 - protein, 11 aa, synthetic construct
  source 1..11: note = Ma7A07_CDR1
SGFTLGDYTLG

SEQ ID NO: 95 - protein, 15 aa, synthetic construct
  source 1..15: note = Ma7A07_CDR2
SSIASSALSIYIADS

SEQ ID NO: 96 - protein, 16 aa, synthetic construct
  source 1..16: note = Ma7A07_CDR3
RGVDSWRWVPSAMDLW

SEQ ID NO: 97 - protein, 123 aa, synthetic construct
  source 1..123: note = VHH_Ma7A08
QVQLVESGGGLVQPGGSLTLSCAASGFTLGDYTLGWFRQAPGKQREGVSSIASSVLSVYIADSVKGRFTISRDDAKNTIYLHMNNLKPEDTGVYYCARGVDSWRWVPSAMDLWGKGTLVTVSS

SEQ ID NO: 98 - protein, 11 aa, synthetic construct
  source 1..11: note = Ma7A08_CDR1
SGFTLGDYTLG

SEQ ID NO: 99 - protein, 15 aa, synthetic construct
  source 1..15: note = Ma7A08_CDR2
SSIASSVLSVYIADS

SEQ ID NO: 100 - protein, 16 aa, synthetic construct
  source 1..16: note = Ma7A08_CDR3
RGVDSWRWVPSAMDLW

SEQ ID NO: 101 - protein, 123 aa, synthetic construct
  source 1..123: note = VHH_Ma7B03
QVQLVESGGGLVQPGGSLRLSCAASGFTLSNYYVGWFRQAPGKQREGVSSIGSSDLSIYIADSVKGRFTISRDNAKNTIYLHMNNLKPDDTGVYYCARGTDSWRWVPSAMDLWGKGTQVTVSS

SEQ ID NO: 102 - protein, 11 aa, synthetic construct
  source 1..11: note = Ma7B03_CDR1
SGFTLSNYYVG

SEQ ID NO: 103 - protein, 15 aa, synthetic construct
  source 1..15: note = Ma7B03_CDR2
SSIGSSDLSIYIADS

SEQ ID NO: 104 - protein, 16 aa, synthetic construct
  source 1..16: note = Ma7B03_CDR3
RGTDSWRWVPSAMDLW

SEQ ID NO: 105 - protein, 123 aa, synthetic construct
  source 1..123: note = VHH_Ma7B12
QVQLVESGGGLVQPGGSLRLSCAASGFTLGDYTLGWFRQAPGKQREGVSSIASSALSIYIADSVKGRFTISRDNAKNTVYLHMNNLKPEDTGVYYCARGIDNWRWVPSAMDLWGKGTQVTVSS

SEQ ID NO: 106 - protein, 11 aa, synthetic construct
  source 1..11: note = Ma7B12_CDR1
SGFTLGDYTLG

SEQ ID NO: 107 - protein, 15 aa, synthetic construct
  source 1..15: note = Ma7B12_CDR2
SSIASSALSIYIADS

SEQ ID NO: 108 - protein, 16 aa, synthetic construct
  source 1..16: note = Ma7B12_CDR3
RGIDNWRWVPSAMDLW

SEQ ID NO: 109 - protein, 125 aa, synthetic construct
  source 1..125: note = VHH_Ma7B01
QVQLVESGGGLVQAGDSLSLSCAASGRTFSNYAMGWFRQAPGKERHFVAVINQIGDSTWYPDFAKGRFTISRDNAKNTLYLQMNSLKPEDTAVYYCAATDPRSYWRIWPHEYGYWGQGTQVTVSS

SEQ ID NO: 110 - protein, 11 aa, synthetic construct
  source 1..11: note = Ma7B01_CDR1
SGRTFSNYAMG

SEQ ID NO: 111 - protein, 15 aa, synthetic construct
  source 1..15: note = Ma7B01_CDR2
AVINQIGDSTWYPDF

SEQ ID NO: 112 - protein, 18 aa, synthetic construct
  source 1..18: note = Ma7B01_CDR3
ATDPRSYWRIWPHEYGYW

SEQ ID NO: 113 - protein, 125 aa, synthetic construct
  source 1..125: note = VHH_Ma7C02
QVQLVESGGGLVQAGGSLRLSCAASGRTFSDYAMGWFRQAAGKDRDFVAVITRSGDSTYYPDSTKGRFTISRDNAKNTMYLQMNSLKPEDTARYYCAATDPTNYWRIWEHEFDYWGQGTQVTVSS

SEQ ID NO: 114 - protein, 11 aa, synthetic construct
  source 1..11: note = Ma7C02_CDR1
SGRTFSDYAMG

SEQ ID NO: 115 - protein, 15 aa, synthetic construct
  source 1..15: note = Ma7C02_CDR2
AVITRSGDSTYYPDS

SEQ ID NO: 116 - protein, 18 aa, synthetic construct
  source 1..18: note = Ma7C02_CDR3
ATDPTNYWRIWEHEFDYW

SEQ ID NO: 117 - protein, 125 aa, synthetic construct
  source 1..125: note = VHH_Ma7E01
QVQLVESGGGSVQAGDSLSLSCVASERTFSNYAMGWFRQAPGKERHFVAVINPIGEETWYPDFAKGRFTISRDNAKNTLYLQMNSLKPEDTAVYYCAATDPRSYWRIWEHEFDYWGQGTQVTVSS

SEQ ID NO: 118 - protein, 11 aa, synthetic construct
  source 1..11: note = Ma7E01_CDR1
SERTFSNYAMG

SEQ ID NO: 119 - protein, 15 aa, synthetic construct
  source 1..15: note = Ma7E01_CDR2
AVINPIGEETWYPDF

SEQ ID NO: 120 - protein, 18 aa, synthetic construct
  source 1..18: note = Ma7E01_CDR3
ATDPRSYWRIWEHEFDYW

SEQ ID NO: 121 - protein, 126 aa, synthetic construct
  source 1..126: note = VHH_Ma7F02
QVQLVESGGGLVQAGGSLRLSCTVSGSIDSLHTMGWFRQAPGKKRDFVAVVSWSGGNTYYPDYAKGRFTISRDNTKNTVYLQMNSLKPEDTAIYYCAAESGSGNYWKIWEHEFDSWGQGTQVTVSS

SEQ ID NO: 122 - protein, 11 aa, synthetic construct
  source 1..11: note = Ma7F02_CDR1
SGSIDSLHTMG

SEQ ID NO: 123 - protein, 15 aa, synthetic construct
  source 1..15: note = Ma7F02_CDR2
AVVSWSGGNTYYPDY

SEQ ID NO: 124 - protein, 19 aa, synthetic construct
  source 1..19: note = Ma7F02_CDR3
AESGSGNYWKIWEHEFDSW

SEQ ID NO: 125 - protein, 126 aa, synthetic construct
  source 1..126: note = VHH_Ma7D06
QVQLVESGGGLVQAGGSLRLSCAASGSISGIDTMAWFRQIPGKDREFVAVIKWAAGSTWYPDFVKGRFTVSRDNAKNMVYLQMDSVKPEDTAIYYCAAAAGEKYYYRLFPYEYDYWGQGTQVTVSS

SEQ ID NO: 126 - protein, 11 aa, synthetic construct
  source 1..11: note = Ma7D06_CDR1
SGSISGIDTMA

SEQ ID NO: 127 - protein, 15 aa, synthetic construct
  source 1..15: note = Ma7D06_CDR2
AVIKWAAGSTWYPDF

SEQ ID NO: 128 - protein, 19 aa, synthetic construct
  source 1..19: note = Ma7D06_CDR3
AAAGEKYYYRLFPYEYDYW

SEQ ID NO: 129 - protein, 124 aa, synthetic construct
  source 1..124: note = VHH_Ma7C11
QVQLVESGGGLVRAGGSLRLSCAASGSISSVNGMGWFRQAPGKERLFVAQVSLLDSSTYYADSVKGRFTISRDDAKNTMYLQMNNVRPEETAVYYCAATKLRIGTAFSSEYDYWGQGTQVTVSS

SEQ ID NO: 130 - protein, 11 aa, synthetic construct
  source 1..11: note = Ma7C11_CDR1
SGSISSVNGMG

SEQ ID NO: 131 - protein, 15 aa, synthetic construct
  source 1..15: note = Ma7C11_CDR2
AQVSLLDSSTYYADS

SEQ ID NO: 132 - protein, 17 aa, synthetic construct
  source 1..17: note = Ma7C11_CDR3
ATKLRIGTAFSSEYDYW

SEQ ID NO: 133 - protein, 126 aa, synthetic construct
  source 1..126: note = VHH_Ma8E03
QVQLVESGGGLVHPGGSLRLSCAASGSSLDHYVIGWFRQVPGKEREGVSCISRSGGSTNYADSVKGRFTVSRDNVKNMVYLQMNSLEPEDSAEYYCAAQRNLGNFCVLGWLEYDDWGQGTQVTVSS

SEQ ID NO: 134 - protein, 11 aa, synthetic construct
  source 1..11: note = Ma8E03_CDR1
SGSSLDHYVIG

SEQ ID NO: 135 - protein, 15 aa, synthetic construct
  source 1..15: note = Ma8E03_CDR2
SCISRSGGSTNYADS

SEQ ID NO: 136 - protein, 19 aa, synthetic construct
  source 1..19: note = Ma8E03_CDR3
AQRNLGNFCVLGWLEYDDW

SEQ ID NO: 137 - protein, 126 aa, synthetic construct
  source 1..126: note = VHH_Ma8G02
QVQLVESGGGLVLPGGSLRLSCAASGSSLDHYVIGWFRQYPGKEREGVSCISRSGGSTNYADSVKGRFTVSRDNVKNMVYLQMNSLEPEDSAEYYCAAQRNLGNFCVLGWVEYDDWGQGTQVTVSS

SEQ ID NO: 138 - protein, 11 aa, synthetic construct
  source 1..11: note = Ma8G02_CDR1
SGSSLDHYVIG

SEQ ID NO: 139 - protein, 15 aa, synthetic construct
  source 1..15: note = Ma8G02_CDR2
SCISRSGGSTNYADS

SEQ ID NO: 140 - protein, 19 aa, synthetic construct
  source 1..19: note = Ma8G02_CDR3
AQRNLGNFCVLGWVEYDDW

SEQ ID NO: 141 - protein, 125 aa, synthetic construct
  source 1..125: note = VHH_Ma8H03
QVQLVESGGGLVHPGGSLRLSCAASGSSLDHYVIGWFRQVPGKQREGISCISSGGSTNYADSVKGRFTVSRDNVKSTVYLQMNSLAPDDSAEYYCAAQRNLGNFCVLGWLEYDDWGQGTQVTVSS

SEQ ID NO: 142 - protein, 11 aa, synthetic construct
  source 1..11: note = Ma8H03_CDR1
SGSSLDHYVIG

SEQ ID NO: 143 - protein, 14 aa, synthetic construct
  source 1..14: note = Ma8H03_CDR2
SCISSGGSTNYADS

SEQ ID NO: 144 - protein, 19 aa, synthetic construct
  source 1..19: note = Ma8H03_CDR3
AQRNLGNFCVLGWLEYDDW

SEQ ID NO: 145 - protein, 126 aa, synthetic construct
  source 1..126: note = VHH_Ma8A05
QVQLVESGGGLVQPGGSLRLSCAASPASGFTLDLYTIAWFLQAPGKEREGVSAISLSDEITYYSDAVKGRFTISRDSAKNTVFLQMDRLKPEDTGVYYCAIGAFDFILKEADADYWGQGTQVTVSS

SEQ ID NO: 146 - protein, 14 aa, synthetic construct
  source 1..14: note = Ma8A05_CDR1
SPASGFTLDLYTIA

SEQ ID NO: 147 - protein, 15 aa, synthetic construct
  source 1..15: note = Ma8A05_CDR2
SAISLSDEITYYSDA

SEQ ID NO: 148 - protein, 16 aa, synthetic construct
  source 1..16: note = Ma8A05_CDR3
IGAFDFILKEADADYW

SEQ ID NO: 149 - protein, 126 aa, synthetic construct
  source 1..126: note = VHH_Ma8D05
QVQLVESGGGLVQPGGSLRLSCAASPASGFTLDLYTIAWFLQAPGKEREGVSAISLSDEITYYSDTVKGRFTISRDSAKNTVFLQMDRLKPEDTGVYYCAIGAFDFILKEADADYWGQGTQVTVSS

SEQ ID NO: 150 - protein, 14 aa, synthetic construct
  source 1..14: note = Ma8D05_CDR1
SPASGFTLDLYTIA

SEQ ID NO: 151 - protein, 15 aa, synthetic construct
  source 1..15: note = Ma8D05_CDR2
SAISLSDEITYYSDT

SEQ ID NO: 152 - protein, 16 aa, synthetic construct
  source 1..16: note = Ma8D05_CDR3
IGAFDFILKEADADYW

SEQ ID NO: 153 - protein, 117 aa, synthetic construct
  source 1..117: note = VHH_Ma8D07
QVQLVESGGGLVQPGGSLRLSCAASESIYKLNAMGWYRQAPGKELELVTTISSGGSTFYTDPVKGRFTISTDNAKNTVYLQMRSLKPEDTAMYYCAANPTYNHYSARGQGTQVTVSS

SEQ ID NO: 154 - protein, 11 aa, synthetic construct
  source 1..11: note = Ma8D07_CDR1
SESIYKLNAMG

SEQ ID NO: 155 - protein, 14 aa, synthetic construct
  source 1..14: note = Ma8D07_CDR2
TTISSGGSTFYTDP

SEQ ID NO: 156 - protein, 11 aa, synthetic construct
  source 1..11: note = Ma8D07_CDR3
ANPTYNHYSAR

SEQ ID NO: 157 - protein, 117 aa, synthetic construct
  source 1..117: note = VHH_Ma8D08
QVQLVESGGGFVQAGGSLRLSCAASESIYKLNAMGWYRQAPGKELELVTTISSGGSTFYTDPVKGRFTISTDNAKNTVYLQMRSLKPEDTAMYYCAANPTYNHYSARGQGTQVTVSS

SEQ ID NO: 158 - protein, 11 aa, synthetic construct
  source 1..11: note = Ma8D08_CDR1
SESIYKLNAMG

SEQ ID NO: 159 - protein, 14 aa, synthetic construct
  source 1..14: note = Ma8D08_CDR2
TTISSGGSTFYTDP

SEQ ID NO: 160 - protein, 11 aa, synthetic construct
  source 1..11: note = Ma8D08_CDR3
ANPTYNHYSAR

SEQ ID NO: 161 - protein, 123 aa, synthetic construct
  source 1..123: note = VHH_Bm28F09
QVQLVESGGGLVEPGGSLTLSCAASGFTSKNYYIGWFRQAPGKYREGVASIGASDGSLYIADSVKGRFTISSDNAKNTVYLHPRNLKPEDSGVYYCATGRDSWRWVPSAMDYWGKGIQVTVSS

SEQ ID NO: 162 - protein, 11 aa, synthetic construct
  source 1..11: note = Bm28F09_CDR1
SGFTSKNYYIG

SEQ ID NO: 163 - protein, 15 aa, synthetic construct
  source 1..15: note = Bm28F09_CDR2
ASIGASDGSLYIADS

SEQ ID NO: 164 - protein, 16 aa, synthetic construct
  source 1..16: note = Bm28F09_CDR3
TGRDSWRWVPSAMDYW

SEQ ID NO: 165 - protein, 123 aa, synthetic construct
  source 1..123: note = VHH_Bm28H01
QVQLVESGGGLVQPGGSLTLSCAASGFTLGDRTLGWFRQVAGKQREGVASIASGVLSAYIADSVKGRFTISRDDAKNTIYLHMNNLKPDDTGVYYCARGVDSWRWVPSTMDLWGKGILVTVSS

SEQ ID NO: 166 - protein, 11 aa, synthetic construct
  source 1..11: note = Bm28H01_CDR1
SGFTLGDRTLG

SEQ ID NO: 167 - protein, 15 aa, synthetic construct
  source 1..15: note = Bm28H01_CDR2
ASIASGVLSAYIADS

SEQ ID NO: 168 - protein, 16 aa, synthetic construct
  source 1..16: note = Bm28H01_CDR3
RGVDSWRWVPSTMDLW

SEQ ID NO: 169 - protein, 126 aa, synthetic construct
  source 1..126: note = VHH_Ma31A12
QVQLVESGGGLVQPGGSLRLSCAASAASGFTLDLYTIAWFLQAPGKEREGVSAISLSDEITYYSDAVKGRFTISRDSAKNTVFLQMDRLKPEDTGVYYCAIGAFDFILKEVDADYWGQGTQVTVSS

SEQ ID NO: 170 - protein, 14 aa, synthetic construct
  source 1..14: note = Ma31A12_CDR1
SAASGFTLDLYTIA

SEQ ID NO: 171 - protein, 15 aa, synthetic construct
  source 1..15: note = Ma31A12_CDR2
SAISLSDEITYYSDA

SEQ ID NO: 172 - protein, 16 aa, synthetic construct
  source 1..16: note = Ma31A12_CDR3
IGAFDFILKEVDADYW

SEQ ID NO: 173 - protein, 126 aa, synthetic construct
  source 1..126: note = VHH_Ma31B06
QVQLVQSGGGLVQPGGTLRLSCAASPASGFTLDLYTIAWFLQAPGKEREGVSAISLSDEITYYSDAVKGRFTISRDSAKNTVFLQMDRLKPEDTGVYYCAIGAFDFILKEADADYWGQGTQVTVSS

SEQ ID NO: 174 - protein, 14 aa, synthetic construct
  source 1..14: note = Ma31B06_CDR1
SPASGFTLDLYTIA

SEQ ID NO: 175 - protein, 15 aa, synthetic construct
  source 1..15: note = Ma31B06_CDR2
SAISLSDEITYYSDA

SEQ ID NO: 176 - protein, 16 aa, synthetic construct
  source 1..16: note = Ma31B06_CDR3
IGAFDFILKEADADYW

SEQ ID NO: 177 - protein, 121 aa, synthetic construct
  source 1..121: note = VHH_Bm28C04
QVQLVESGGGSVQPGNSLRLSCKVSGRTFNSYALGWFRRRPGDQRDFVASIIRSTGGTSYADSVKGRFTISYDNVQNTVDLQMNSLEPEDTAIYYCAGGDGHIYAFGYDYWGQGTQVTVSS

SEQ ID NO: 178 - protein, 11 aa, synthetic construct
  source 1..11: note = Bm28C04_CDR1
SGRTFNSYALG

SEQ ID NO: 179 - protein, 15 aa, synthetic construct
  source 1..15: note = Bm28C04_CDR2
ASIIRSTGGTSYADS

SEQ ID NO: 180 - protein, 14 aa, synthetic construct
  source 1..14: note = Bm28C04_CDR3
GGDGHIYAFGYDYW

SEQ ID NO: 181 - protein, 121 aa, synthetic construct
  source 1..121: note = VHH_Bm28H07
QVQLVESGGGSVQPGNSLRLSCKVSGRTFNSYALGWFRRRPGDQRDFVASIIRSTGGTSYADSVKGRFTISYDNVQNTVDLQMSSLEPEDTAIYYCAGGDGHIYAFGYDYWGQGTQVTVSS

SEQ ID NO: 182 - protein, 11 aa, synthetic construct
  source 1..11: note = Bm28H07_CDR1
SGRTFNSYALG

SEQ ID NO: 183 - protein, 15 aa, synthetic construct
  source 1..15: note = Bm28H07_CDR2
ASIIRSTGGTSYADS

SEQ ID NO: 184 - protein, 14 aa, synthetic construct
  source 1..14: note = Bm28H07_CDR3
GGDGHIYAFGYDYW

SEQ ID NO: 185 - protein, 123 aa, synthetic construct
  source 1..123: note = VHH_Bm28C09
QVQLVESGGSVVQAGGSLRLSCTASGRNFNSYAMGWFRRPPGEQRDFIAAIIRSTGKTTYADSDSVKGRFTISKDSSGNTVYLQMNNLKPEDTAIYYCAGGDAGPYAFGYDYWGQGTQVTVSS

SEQ ID NO: 186 - protein, 11 aa, synthetic construct
  source 1..11: note = Bm28C09_CDR1
SGRNFNSYAMG

SEQ ID NO: 187 - protein, 17 aa, synthetic construct
  source 1..17: note = Bm28C09_CDR2
AAIIRSTGKTTYADSDS

SEQ ID NO: 188 - protein, 14 aa, synthetic construct
  source 1..14: note = Bm28C09_CDR3
GGDAGPYAFGYDYW

SEQ ID NO: 189 - protein, 123 aa, synthetic construct; identical to SEQ ID NO: 185
  source 1..123: note = VHH_Bm28H12

SEQ ID NO: 190 - protein, 11 aa, synthetic construct
  source 1..11: note = Bm28H12_CDR1
SGRNFNSYAMG

SEQ ID NO: 191 - protein, 17 aa, synthetic construct
  source 1..17: note = Bm28H12_CDR2
AAIIRSTGKTTYADSDS

SEQ ID NO: 192 - protein, 14 aa, synthetic construct
  source 1..14: note = Bm28H12_CDR3
GGDAGPYAFGYDYW

SEQ ID NO: 193 - protein, 125 aa, synthetic construct
  source 1..125: note = VHH_Bm28A12
QVQLVESGGGLVQAGGSLRLSCVVSGRALSSYNLAWFRQSPGKEREWIATIMPSADKAHYPDFLEGRFTISGDNTENTLYLQMNSLKPEDTAIYYCAAREPSYYHALFEYEYNLWGQGTQVTVSS

SEQ ID NO: 194 - protein, 11 aa, synthetic construct
  source 1..11: note = Bm28A12_CDR1
SGRALSSYNLA

SEQ ID NO: 195 - protein, 15 aa, synthetic construct
  source 1..15: note = Bm28A12_CDR2
ATIMPSADKAHYPDF

SEQ ID NO: 196 - protein, 17 aa, synthetic construct
  source 1..17: note = Bm28A12_CDR3
REPSYYHALFEYEYNLW

SEQ ID NO: 197 - protein, 518 aa, synthetic construct
  source 1..518: note = Ma7A07-Bm29C02-Fc fusion
ETGGSQVQLVESGGGLVQPGGSLRLSCAASGFTLGDYTLGWFRQAPGKQREGVSSIASSALSIYIADSVKGRFTISRDDAKNTIYLHMNNLKPEDTGVYYCARGVDSWRWVPSAMDLWGKGTLVTVSSTSTSGEGEGGGEGGSQVQLVESGGGLVQPGGSLRLSCTASGFTLDDWAIGWFRQAPGKEREGVSCTSSRERSSYYRDSVKGRFTISRDSTSNTVYLQMNELTLEDTAVYYCAADPQPYPCSLGQLGRYTTWGQGTQVTVSSGTENLYFQGKSCDKTHTCPPCPAPELLGGPSVFLFPPKPKDTLMISRTPEVTCVVVDVSHEDPEVKFNWYVDGVEVHNAKTKPREEQYNSTYRVVSVLTVLHQDWLNGKEYKCKVSNKALPAPIEKTISKAKGQPREPQVYTLPPSRDELTKNQVSLTCLVKGFYPSDIAVEWESNGQPENNYKATPPVLDSDGSFFLYSKLTVDKSRWQQGNVFSCSVMHEALHNHYTQKSLSLSPGKSGTSHHHHHH